European Patent Specification EP 3 748 001 B1, published May 13, 2026. Title: Peptide Library and Uses Thereof. Applicant: Daiichi Sankyo Co., Ltd. The sequence listing filed with the application follows.

SEQUENCE LISTING (35 sequences)

SEQ ID NO: 1 - protein, 17 aa, Artificial Sequence
  Peptide with diversity
  MISC_FEATURE (2)..(8): any amino acid
  MISC_FEATURE (10)..(14): any amino acid
CXXXXXXXCXXXXXPVC

SEQ ID NO: 2 - protein, 17 aa, Artificial Sequence
  Peptide No.1 binding to alpha-chymotripsin
CRTRWGNRCTWQYKPVC

SEQ ID NO: 3 - protein, 17 aa, Artificial Sequence
  Peptide No.2 binding to alpha-chymotripsin
CMRHRRHFCTMVYKPVC

SEQ ID NO: 4 - protein, 17 aa, Artificial Sequence
  Peptide No.6 binding to alpha-chymotripsin
CRRWLLPWCTYKYKPVC

SEQ ID NO: 5 - protein, 17 aa, Artificial Sequence
  Peptide No.7 binding to alpha-chymotripsin
CLWRRHKLCPFKFKPVC

SEQ ID NO: 6 - protein, 17 aa, Artificial Sequence
  Peptide No.12 binding to alpha-chymotripsin
CWRSWRWACPYMYKPVC

SEQ ID NO: 7 - protein, 17 aa, Artificial Sequence
  Peptide No.13 binding to alpha-chymotripsin
CWFFRWRWCNWALKPVC

SEQ ID NO: 8 - protein, 17 aa, Artificial Sequence
  Peptide No.14 binding to alpha-chymotripsin
CSTWRMWGCPWLYKPVC

SEQ ID NO: 9 - protein, 17 aa, Artificial Sequence
  Peptide No.17 binding to alpha-chymotripsin
CWRRWYDRCSFNLKPVC

SEQ ID NO: 10 - DNA, 55 bp, Artificial Sequence
  Fragment 1
gtacccgataaaagcggcttcctgacaggaggccgttttgttttgcagcccacct

SEQ ID NO: 11 - DNA, 136 bp, Artificial Sequence
  Fragment 2
cgcaacgcaattaatgtgagttagctcactcattaggcaccccaggctttacactttatgcttccggctcgtatgttgtgtggaattgtgagcggataacaatttcacacaggaaacagctatgaccatgattacg

SEQ ID NO: 12 - DNA, 309 bp, Artificial Sequence
  Fragment 3
aatttctagataacgagggcaaatcatgaaacaaagcactattgcactggcactcttaccgttgctgtttacccctgtgacgaaagctgctagcgcgaattctgatccgcagtttggtctgtttagcaaatatcgtaccccgaattgtagccagtatcgtctgcctggttgtccgcgtcattttaatccggtttgtggtagcgatatgagcacctatgcaaatgaatgtaccctgtgcatgaaaattcgtgaaggtggccataatattaaaattattcgcaatggtccgtgcgacgcgtctgcggccgc

SEQ ID NO: 13 - DNA, 57 bp, Artificial Sequence
  Fragment 5
ctgtgaagtgaaaaatggcgcacattgtgcgacattttttttgtctgccgtttaatc

SEQ ID NO: 14 - DNA, 192 bp, Homo sapiens
  CDS (1)..(192)
gatccgcagtttggtctgtttagcaaatatcgtaccccgaattgtagccagtatcgtctgcctggttgtccgcgtcattttaatccggtttgtggtagcgatatgagcacctatgcaaatgaatgtaccctgtgcatgaaaattcgtgaaggtggccataatattaaaattattcgcaatggtccgtgctaa

SEQ ID NO: 15 - protein, 63 aa, Homo sapiens
DPQFGLFSKYRTPNCSQYRLPGCPRHFNPVCGSDMSTYANECTLCMKIREGGHNIKIIRNGPC

SEQ ID NO: 16 - DNA, 1916 bp, Artificial
  A template DNA for PCR comprising Fragments 1 to 5
gaagagcgcccaatacgcaaaccgcctctccccgcgcgttggccgattcattaatgcagctggcacgacaggtttcccgactggaaagcgggcagtgagcggtacccgataaaagcggcttcctgacaggaggccgttttgttttgcagcccacctcaacgcaattaatgtgagttagctcactcattaggcaccccaggctttacactttatgcttccggctcgtatgttgtgtggaattgtgagcggataacaatttcacacaggaaacagctatgaccatgattacgaatttctagataacgagggcaaatcatgaaacaaagcactattgcactggcactcttaccgttgctgtttacccctgtgacgaaagctgctagcgcgaattctgatccgcagtttggtctgtttagcaaatatcgtaccccgaattgtagccagtatcgtctgcctggttgtccgcgtcattttaatccggtttgtggtagcgatatgagcacctatgcaaatgaatgtaccctgtgcatgaaaattcgtgaaggtggccataatattaaaattattcgcaatggtccgtgcgacgcgtctgcggccgcataggcaggtgcatctggcggtggttctggcgcaaccgttgaaagttgtttagcaaaaccccatacagaaaattcatttactaacgtctggaaagacgacaaaactttagatcgttacgctaactatgagggctgtctgtggaatgctacaggcgttgtggtttgtactggtgacgaaactcagtgttacggtacatgggttcctattgggcttgctatccctgaaaatgagggtggtggctctgagggtggcggttctgagggtggcggttctgagggtggcggtactaaacctcctgagtacggtgatacacctattccgggctatacttatatcaaccctctcgacggcacttatccgcctggtactgagcaaaaccccgctaatcctaatccttctcttgaggagtctcagcctcttaatactttcatgtttcagaataataggttccgaaataggcagggtgcattaactgtttatacgggcactgttactcaaggcactgaccccgttaaaacttattaccagtacactcctgtatcatcaaaagccatgtatgacgcttactggaacggtaaattcagagactgcgctttccattctggctttaatgaggatccattcgtttgtgaatatcaaggccaatcgtctgacctgcctcaacctcctgtcaatgctggcggcggctctggtggtggttctggtggcggctctgagggtggcggctctgagggtggcggttctgagggtggcggctctgagggtggcggttccggtggcggctccggttccggtgattttgattatgaaaaaatggcaaacgctaataagggggctatgaccgaaaatgccgatgaaaacgcgctacagtctgacgctaaaggcaaacttgattctgtcgctactgattacggtgctgctatcgatggtttcattggtgacgtttccggccttgctaatggtaatggtgctactggtgattttgctggctctaattcccaaatggctcaagtcggtgacggtgataattcacctttaatgaataatttccgtcaatatttaccttctttgcctcagtcggttgaatgtcgcccttatgtctttggcgctggtaaaccatatgaattttctattgattgtgacaaaataaacttattccgtggtgtctttgcgtttcttttatatgttgccacctttatgtatgtattttcgacgtttgctaacatactgcgtaataaggagtcttaatagtacctgtgaagtgaaaaatggcgcacattgtgcgacattttttttgtctgccgtttaatgaattc

SEQ ID NO: 17 - DNA, 39 bp, Artificial Sequence
  Primer 1
aaaaaacgcgtctgcggccgcatagggtagcgaaaacct

SEQ ID NO: 18 - DNA, 40 bp, Artificial Sequence
  Primer 2
aaaaaggcgccattcgccattcaggctgcgcaactgttgg

SEQ ID NO: 19 - DNA, 35 bp, Artificial Sequence
  Primer 1'
aaaagaagagcgcccaatacgcaaaccgcctctcc

SEQ ID NO: 20 - DNA, 39 bp, Artificial Sequence
  Primer 2'
aaaaagaattcattaaacggcagacaaaaaaaatgtcgc

SEQ ID NO: 21 - DNA, 38 bp, Artificial Sequence
  Primer 3
gcggccgcatagggtagcgaaaacctgtattttcagag

SEQ ID NO: 22 - DNA, 42 bp, Artificial Sequence
  Primer 4
gctaaacaactttcaacggtgctaccgctctgaaaatacagg

SEQ ID NO: 23 - DNA, 27 bp, Artificial Sequence
  Primer 5
accgttgaaagttgtttagcaaaaccc

SEQ ID NO: 24 - DNA, 28 bp, Artificial Sequence
  Primer 6
cattaaagccagaatggaaagcgcagtc

SEQ ID NO: 25 - DNA, 29 bp, Artificial Sequence
  Primer alpha
aacacgcgtctgcggccgcatagggtagc

SEQ ID NO: 26 - DNA, 31 bp, Artificial Sequence
  Primer beta
aacggatcctcattaaagccagaatggaaag

SEQ ID NO: 27 - DNA, 23 bp, Artificial Sequence
  Primer 7
ggtagcgatatgagcacctatgc

SEQ ID NO: 28 - DNA, 19 bp, Artificial Sequence
  Primer 8
gcacggaccattgcgaata

SEQ ID NO: 29 - DNA, 37 bp, Artificial Sequence
  Primer 9
gtttggtctgtttagcaaatatcgtaccccgaattgt

SEQ ID NO: 30 - DNA, 19 bp, Artificial Sequence
  Primer 10
gcacggaccattgcgaata

SEQ ID NO: 31 - DNA, 44 bp, Artificial Sequence
  Primer 11
aaagaattctgatccgcagtttggtctgtttagcaaataatcgt

SEQ ID NO: 32 - DNA, 38 bp, Artificial Sequence
  Primer 12
aaaggcgcgccgcacggaccattgcgaataattttaat

SEQ ID NO: 33 - DNA, 37 bp, Artificial Sequence
  Primer 13
aaaggatccgcgaattcatgaccgagtacaagcccac

SEQ ID NO: 34 - DNA, 40 bp, Artificial Sequence
  Primer 14
aaactcgagttatgcggccgctcaggcaccgggcttgcgg

SEQ ID NO: 35 - DNA, 27 bp, Artificial Sequence
  Primer 15
gttctggttctggccatatgcaccatc